European Patent Application EP 4 339 615 A2, published March 20, 2024. Title: ANTI-PD-1 ANTIBODIES. Applicant: SHANGHAI HENLIUS BIOTECH, INC. Application EP, filed September 9, 2017. The sequence listing filed with the application follows.

SEQUENCE LISTING (34 sequences)

SEQ ID NO: 1 - DNA, 651 bp, synthetic construct
  misc_feature 1..651: note = Description of Artificial Sequence: Synthetic polynucleotide
  source 1..651: mol_type = other DNA
cagctcgaggatattgtgatgacccagtctcacaaattcatgtccacatcagtaggagacagggtcagcatcacctgcaaggccagtcaggatgtgactactgctgtagcctggtatcaacaaaaaccagggcaatctcctaaactactgatttactgggcatccacccggcacactggagtccctgatcgcttcacaggcagtggatctgggacagattatactctcaccatcaacagtgtgcaggctgaagacctggcactttattactgtcagcaacattacactattccgtggacgttcggtggaggcaccaagctggaaatcaaacgtactgtggctgcaccatctgtcttcatcttcccgccatctgatgagcagttgaaatctggaactgcctctgttgtgtgcctgctgaataacttctatcccagagaggccaaagtacagtggaaggtggataacgccctccaatcgggtaactcccaggagagtgtcacagagcaggacagcaaggacagcacctacagcctcagcagcaccctgacgctgagcaaagcagactacgagaaacacaaagtctacgcctgcgaagtcacccatcagggcctgagctcgcccgtcacaaagagcttcaacaggggagagtgt

SEQ ID NO: 2 - protein, 217 aa, synthetic construct
  REGION 1..217: note = Description of Artificial Sequence: Synthetic polypeptide
QLEDIVMTQSHKFMSTSVGDRVSITCKASQDVTTAVAWYQQKPGQSPKLLIYWASTRHTGVPDRFTGSGSGTDYTLTINSVQAEDLALYYCQQHYTIPWTFGGGTKLEIKRTVAAPSVFIFPPSDEQLKSGTASVVCLLNNFYPREAKVQWKVDNALQSGNSQESVTEQDSKDSTYSLSSTLTLSKADYEKHKVYACEVTHQGLSSPVTKSFNRGEC

SEQ ID NO: 3 - DNA, 1329 bp, synthetic construct
  misc_feature 1..1329: note = Description of Artificial Sequence: Synthetic polynucleotide
  source 1..1329: mol_type = other DNA
gaagtgatgttggtggagtctgggggaggcttagtgaagcctggagggtccctgaaactctcatgtgcagcctctggattcactttcagtaactatggcatgtcttgggttcgccagactccggagaagagcctggagtgggtcgcaaccattagtggtggtggtagtaacatctactatccagacagtgtgaaggggcgattcaccatctccagagacaatgccaagaacaacctgttcctgcaaatgagcggtctgaggtctgaggacacggccctgtattactgtgtatcgtattactatggaatagacttctggggtcaaggaacctcagtcaccgtctcctcggcctccaccaagggcccatcggtcttcccgctagcaccctgctccaggagcacctccgagagcacagccgccctgggctgcctggtcaaggactacttccccgaaccggtgacggtgtcgtggaactcaggcgccctgaccagcggcgtgcacaccttcccggctgtcctacagtcctcaggactctactccctcagcagcgtggtgaccgtgccctccagcagcttgggcacgaagacctacacctgcaacgtagatcacaagcccagcaacaccaaggtggacaagagagttgagtccaaatatggtcccccatgcccaccatgcccagcacctgagttcctggggggaccatcagtcttcctgttccccccaaaacccaaggacactctcatgatctcccggacccctgaggtcacgtgcgtggtggtggacgtgagccaggaagaccccgaggtccagttcaactggtacgtggatggcgtggaggtgcataatgccaagacaaagccgcgggaggagcagttcaacagcacgtaccgtgtggtcagcgtcctcaccgtcctgcaccaggactggctgaacggcaaggagtacaagtgcaaggtctccaacaaaggcctcccgtcctccatcgagaaaaccatctccaaagccaaagggcagccccgagagccacaggtgtacaccctgcccccatcccaggaggagatgaccaagaaccaggtcagcctgacctgcctggtcaaaggcttctaccccagcgacatcgccgtggagtgggagagcaatgggcagccggagaacaactacaagaccacgcctcccgtgctggactccgacggctccttcttcctctacagcaggctaaccgtggacaagagcaggtggcaggaggggaatgtcttctcatgctccgtgatgcatgaggctctgcacaaccactacacacagaagagcctctccctgtctctgggtaaa

SEQ ID NO: 4 - protein, 443 aa, synthetic construct
  REGION 1..443: note = Description of Artificial Sequence: Synthetic polypeptide
EVMLVESGGGLVKPGGSLKLSCAASGFTFSNYGMSWVRQTPEKSLEWVATISGGGSNIYYPDSVKGRFTISRDNAKNNLFLQMSGLRSEDTALYYCVSYYYGIDFWGQGTSVTVSSASTKGPSVFPLAPCSRSTSESTAALGCLVKDYFPEPVTVSWNSGALTSGVHTFPAVLQSSGLYSLSSVVTVPSSSLGTKTYTCNVDHKPSNTKVDKRVESKYGPPCPPCPAPEFLGGPSVFLFPPKPKDTLMISRTPEVTCVVVDVSQEDPEVQFNWYVDGVEVHNAKTKPREEQFNSTYRVVSVLTVLHQDWLNGKEYKCKVSNKGLPSSIEKTISKAKGQPREPQVYTLPPSQEEMTKNQVSLTCLVKGFYPSDIAVEWESNGQPENNYKTTPPVLDSDGSFFLYSRLTVDKSRWQEGNVFSCSVMHEALHNHYTQKSLSLSLGK

SEQ ID NO: 5 - DNA, 642 bp, synthetic construct
  misc_feature 1..642: note = Description of Artificial Sequence: Synthetic polynucleotide
  source 1..642: mol_type = other DNA
gacatccagatgacccagtctccatcctccctgtctgcatctgtaggagacagagtcaccatcacttgcaaggccagtcaggatgtgactactgctgtagcctggtatcagcagaaaccagggaaagcccctaagctcctgatctattgggcatccacccggcacactggggtcccatcaaggttcagtggcagtggatctgggacagatttcactctcaccatcagcagtctgcaacctgaagattttgcaacttactactgtcagcaacattacactattccgtggacgttcggtggaggcaccaagctggaaatcaaacgtactgtggctgcaccatctgtcttcatcttcccgccatctgatgagcagttgaaatctggaactgcctctgttgtgtgcctgctgaataacttctatcccagagaggccaaagtacagtggaaggtggataacgccctccaatcgggtaactcccaggagagtgtcacagagcaggacagcaaggacagcacctacagcctcagcagcaccctgacgctgagcaaagcagactacgagaaacacaaagtctacgcctgcgaagtcacccatcagggcctgagctcgcccgtcacaaagagcttcaacaggggagagtgt

SEQ ID NO: 6 - protein, 214 aa, synthetic construct
  REGION 1..214: note = Description of Artificial Sequence: Synthetic polypeptide
DIQMTQSPSSLSASVGDRVTITCKASQDVTTAVAWYQQKPGKAPKLLIYWASTRHTGVPSRFSGSGSGTDFTLTISSLQPEDFATYYCQQHYTIPWTFGGGTKLEIKRTVAAPSVFIFPPSDEQLKSGTASVVCLLNNFYPREAKVQWKVDNALQSGNSQESVTEQDSKDSTYSLSSTLTLSKADYEKHKVYACEVTHQGLSSPVTKSFNRGEC

SEQ ID NO: 7 - DNA, 1329 bp, synthetic construct
  misc_feature 1..1329: note = Description of Artificial Sequence: Synthetic polynucleotide
  source 1..1329: mol_type = other DNA
caggtgcagctggtggagtctgggggaggcttggtcaagcctggagggtccctgagactctcctgtgcagcctctggattcactttcagtaactatggcatgtcttggatccgccaggctccagggaaggggctggagtgggtttcaaccattagtggtggtggtagtaacatctactacgcagactctgtgaagggccgattcaccatctccagggacaacgccaagaactcactgtatctgcaaatgaacagcctgagagccgaggacacggctgtgtattactgtgtatcgtattactatggaatagacttctggggtcaaggaacctcagtcaccgtctcctcggcctccaccaagggcccatcggtcttcccgctagcaccctgctccaggagcacctccgagagcacagccgccctgggctgcctggtcaaggactacttccccgaaccggtgacggtgtcgtggaactcaggcgccctgaccagcggcgtgcacaccttcccggctgtcctacagtcctcaggactctactccctcagcagcgtggtgaccgtgccctccagcagcttgggcacgaagacctacacctgcaacgtagatcacaagcccagcaacaccaaggtggacaagagagttgagtccaaatatggtcccccatgcccaccatgcccagcacctgagttcctggggggaccatcagtcttcctgttccccccaaaacccaaggacactctcatgatctcccggacccctgaggtcacgtgcgtggtggtggacgtgagccaggaagaccccgaggtccagttcaactggtacgtggatggcgtggaggtgcataatgccaagacaaagccgcgggaggagcagttcaacagcacgtaccgtgtggtcagcgtcctcaccgtcctgcaccaggactggctgaacggcaaggagtacaagtgcaaggtctccaacaaaggcctcccgtcctccatcgagaaaaccatctccaaagccaaagggcagccccgagagccacaggtgtacaccctgcccccatcccaggaggagatgaccaagaaccaggtcagcctgacctgcctggtcaaaggcttctaccccagcgacatcgccgtggagtgggagagcaatgggcagccggagaacaactacaagaccacgcctcccgtgctggactccgacggctccttcttcctctacagcaggctaaccgtggacaagagcaggtggcaggaggggaatgtcttctcatgctccgtgatgcatgaggctctgcacaaccactacacacagaagagcctctccctgtctctgggtaaa

SEQ ID NO: 8 - protein, 443 aa, synthetic construct
  REGION 1..443: note = Description of Artificial Sequence: Synthetic polypeptide
QVQLVESGGGLVKPGGSLRLSCAASGFTFSNYGMSWIRQAPGKGLEWVSTISGGGSNIYYADSVKGRFTISRDNAKNSLYLQMNSLRAEDTAVYYCVSYYYGIDFWGQGTSVTVSSASTKGPSVFPLAPCSRSTSESTAALGCLVKDYFPEPVTVSWNSGALTSGVHTFPAVLQSSGLYSLSSVVTVPSSSLGTKTYTCNVDHKPSNTKVDKRVESKYGPPCPPCPAPEFLGGPSVFLFPPKPKDTLMISRTPEVTCVVVDVSQEDPEVQFNWYVDGVEVHNAKTKPREEQFNSTYRVVSVLTVLHQDWLNGKEYKCKVSNKGLPSSIEKTISKAKGQPREPQVYTLPPSQEEMTKNQVSLTCLVKGFYPSDIAVEWESNGQPENNYKTTPPVLDSDGSFFLYSRLTVDKSRWQEGNVFSCSVMHEALHNHYTQKSLSLSLGK

SEQ ID NO: 9 - protein, 11 aa, synthetic construct
  REGION 1..11: note = Description of Artificial Sequence: Synthetic peptide
KASQDVTTAVA

SEQ ID NO: 10 - protein, 7 aa, synthetic construct
  REGION 1..7: note = Description of Artificial Sequence: Synthetic peptide
WASTRHT

SEQ ID NO: 11 - protein, 9 aa, synthetic construct
  REGION 1..9: note = Description of Artificial Sequence: Synthetic peptide
QQHYTIPWT

SEQ ID NO: 12 - protein, 9 aa, synthetic construct
  REGION 1..9: note = Description of Artificial Sequence: Synthetic peptide
FTFSNYGMS

SEQ ID NO: 13 - protein, 10 aa, synthetic construct
  REGION 1..10: note = Description of Artificial Sequence: Synthetic peptide
TISGGGSNIY

SEQ ID NO: 14 - protein, 9 aa, synthetic construct
  REGION 1..9: note = Description of Artificial Sequence: Synthetic peptide
VSYYYGIDF

SEQ ID NO: 15 - protein, 11 aa, synthetic construct
  REGION 1..11: note = Description of Artificial Sequence: Synthetic peptide
KASTDVTTAVA

SEQ ID NO: 16 - protein, 7 aa, synthetic construct
  REGION 1..7: note = Description of Artificial Sequence: Synthetic peptide
WASLRHT

SEQ ID NO: 17 - protein, 9 aa, synthetic construct
  REGION 1..9: note = Description of Artificial Sequence: Synthetic peptide
QQHYGIPWT

SEQ ID NO: 18 - protein, 9 aa, synthetic construct
  REGION 1..9: note = Description of Artificial Sequence: Synthetic peptide
FRFSNYGMS

SEQ ID NO: 19 - protein, 10 aa, synthetic construct
  REGION 1..10: note = Description of Artificial Sequence: Synthetic peptide
TISGGGSNAY

SEQ ID NO: 20 - protein, 9 aa, synthetic construct
  REGION 1..9: note = Description of Artificial Sequence: Synthetic peptide
TSYYYGIDF

SEQ ID NO: 21 - protein, 11 aa, synthetic construct
  REGION 1..11: note = Description of Artificial Sequence: Synthetic peptide
KAKQDVTTAVA

SEQ ID NO: 22 - protein, 9 aa, synthetic construct
  REGION 1..9: note = Description of Artificial Sequence: Synthetic peptide
QQHYWIPWT

SEQ ID NO: 23 - protein, 9 aa, synthetic construct
  REGION 1..9: note = Description of Artificial Sequence: Synthetic peptide
VSYYYGIDL

SEQ ID NO: 24 - protein, 11 aa, synthetic construct
  REGION 1..11: note = Description of Artificial Sequence: Synthetic peptide
KASQDVTNAVA

SEQ ID NO: 25 - protein, 9 aa, synthetic construct
  REGION 1..9: note = Description of Artificial Sequence: Synthetic peptide
SSYYYGIDL

SEQ ID NO: 26 - protein, 6 aa, synthetic construct
  REGION 1..6: note = Description of Artificial Sequence: Synthetic 6xHis tag
HHHHHH

SEQ ID NO: 27 - protein, 217 aa, synthetic construct; identical to SEQ ID NO: 2
  REGION 1..217: note = Description of Artificial Sequence: Synthetic polypeptide

SEQ ID NO: 28 - protein, 214 aa, synthetic construct; identical to SEQ ID NO: 6
  REGION 1..214: note = Description of Artificial Sequence: Synthetic polypeptide

SEQ ID NO: 29 - protein, 95 aa, Homo sapiens
DIQMTQSPSSLSASVGDRVTITCRASQSISSYLNWYQQKPGKAPKLLIYAASSLQSGVPSRFSGSGSGTDFTLTISSLQPEDFATYYCQQSYSTP

SEQ ID NO: 30 - protein, 214 aa, synthetic construct
  REGION 1..214: note = Description of Artificial Sequence: Synthetic polypeptide
EIVLTQSPATLSLSPGERATLSCRASQSVSSYLAWYQQKPGQAPRLLIYDASNRATGIPARFSGSGSGTDFTLTISSLEPEDFAVYYCQQSSNWPRTFGQGTKVEIKRTVAAPSVFIFPPSDEQLKSGTASVVCLLNNFYPREAKVQWKVDNALQSGNSQESVTEQDSKDSTYSLSSTLTLSKADYEKHKVYACEVTHQGLSSPVTKSFNRGEC

SEQ ID NO: 31 - protein, 443 aa, synthetic construct; identical to SEQ ID NO: 4
  REGION 1..443: note = Description of Artificial Sequence: Synthetic polypeptide

SEQ ID NO: 32 - protein, 443 aa, synthetic construct; identical to SEQ ID NO: 8
  REGION 1..443: note = Description of Artificial Sequence: Synthetic polypeptide

SEQ ID NO: 33 - protein, 98 aa, Homo sapiens
QVQLVESGGGLVKPGGSLRLSCAASGFTFSDYYMSWIRQAPGKGLEWVSYISSSGSTIYYADSVKGRFTISRDNAKNSLYLQMNSLRAEDTAVYYCAR

SEQ ID NO: 34 - protein, 439 aa, synthetic construct
  REGION 1..439: note = Description of Artificial Sequence: Synthetic polypeptide
QVQLVESGGGVVQPGRSLRLDCKASGITFSNSGMHWVRQAPGKGLEWVAVIWYDGSKRYYADSVKGRFTISRDNSKNTLFLQMNSLRAEDTAVYYCATNDDYWGQGTLVTVSSSTKGPSVFPLAPCSRSTSESTAALGCLVKDYFPEPVTVSWNSGALTSGVHTFPAVLQSSGLYSLSSVVTVPSSSLGTKTYTCNVDHKPSNTKVDKRVESKYGPPCPPCPAPEFLGGPSVFLFPPKPKDTLMISRTPEVTCVVVDVSQEDPEVQFNWYVDGVEVHNAKTKPREEQFNSTYRVVSVLTVLHQDWLNGKEYKCKVSNKGLPSSIEKTISKAKGQPREPQVYTLPPSQEEMTKNQVSLTCLVKGFYPSDIAVEWESNGQPENNYKTTPPVLDSDGSFFLYSRLTVDKSRWQEGNVFSCSVMHEALHNHYTQKSLSLSLGK